European Patent Application EP 4 137 504 A1, published February 22, 2023. Title: Novel Alpha-Helix Ampiphilic Cell Penetrating Peptides and Use Thereof. Applicant: Seoul National University R&DB Foundation. The sequence listing filed with the application follows.

SEQUENCE LISTING (48 sequences)

SEQ ID NO: 1 - protein, 16 aa, Artificial Sequence
  synthetic peptide
LKKLCKLLKKLCKLAG

SEQ ID NO: 2 - protein, 8 aa, Artificial Sequence
  synthetic peptide
CKLLKKLC

SEQ ID NO: 3 - protein, 10 aa, Artificial Sequence
  synthetic peptide
LCKLLKKLCK

SEQ ID NO: 4 - protein, 12 aa, Artificial Sequence
  synthetic peptide
KLCKLLKKLCKL

SEQ ID NO: 5 - protein, 14 aa, Artificial Sequence
  synthetic peptide
KKLCKLLKKLCKLL

SEQ ID NO: 6 - protein, 16 aa, Artificial Sequence
  synthetic peptide
LKKLCKLLKKLCKLLK

SEQ ID NO: 7 - protein, 18 aa, Artificial Sequence
  synthetic peptide
LLKKLCKLLKKLCKLLKK

SEQ ID NO: 8 - protein, 10 aa, Artificial Sequence
  synthetic peptide
FCKFFKKFCK

SEQ ID NO: 9 - protein, 10 aa, Artificial Sequence
  synthetic peptide
FCRFFRRFCR

SEQ ID NO: 10 - protein, 10 aa, Artificial Sequence
  synthetic peptide
ICRIIRRICR

SEQ ID NO: 11 - protein, 10 aa, Artificial Sequence
  synthetic peptide
LCRLLRRLCR

SEQ ID NO: 12 - protein, 10 aa, Artificial Sequence
  synthetic peptide
ICKIIKKICK

SEQ ID NO: 13 - protein, 10 aa, Artificial Sequence
  synthetic peptide
  MISC_FEATURE (1): X is Npg(neopentylglycine)
  MISC_FEATURE (4)..(5): X is Npg
  MISC_FEATURE (8): X is Npg
XCRXXRRXCR

SEQ ID NO: 14 - protein, 10 aa, Artificial Sequence
  synthetic peptide
LCHLLHHLCH

SEQ ID NO: 15 - protein, 10 aa, Artificial Sequence
  synthetic peptide
VCKVVKKVCK

SEQ ID NO: 16 - protein, 10 aa, Artificial Sequence
  synthetic peptide
FCHFFHHFCH

SEQ ID NO: 17 - protein, 10 aa, Artificial Sequence
  synthetic peptide
  MISC_FEATURE (1): X is Npg
  MISC_FEATURE (4)..(5): X is Npg
  MISC_FEATURE (8): X is Npg
XCKXXKKXCK

SEQ ID NO: 18 - protein, 10 aa, Artificial Sequence
  synthetic peptide
VCHVVHHVCH

SEQ ID NO: 19 - protein, 10 aa, Artificial Sequence
  synthetic peptide
  MISC_FEATURE (1): X is Npg
  MISC_FEATURE (4)..(5): X is Npg
  MISC_FEATURE (8): X is Npg
XCHXXHHXCH

SEQ ID NO: 20 - protein, 10 aa, Artificial Sequence
  synthetic peptide
VCRVVRRVCR

SEQ ID NO: 21 - protein, 10 aa, Artificial Sequence
  synthetic peptide
ICHIIHHICH

SEQ ID NO: 22 - protein, 10 aa, Artificial Sequence
  synthetic peptide
  MISC_FEATURE (1): X is Cha(cyclohexylalanine)
  MISC_FEATURE (4)..(5): X is Cha
  MISC_FEATURE (8): X is Cha
XCKXXKKXCK

SEQ ID NO: 23 - protein, 10 aa, Artificial Sequence
  synthetic peptide
LLRLLRRLCR

SEQ ID NO: 24 - protein, 10 aa, Artificial Sequence
  synthetic peptide
LCRLLRRLLR

SEQ ID NO: 25 - protein, 10 aa, Artificial Sequence
  synthetic peptide
  MISC_FEATURE (3): X is Orn(ornithine)
  MISC_FEATURE (6)..(7): X is Orn
  MISC_FEATURE (10): X is Orn
LCXLLXXLCX

SEQ ID NO: 26 - protein, 10 aa, Artificial Sequence
  synthetic peptide
  MISC_FEATURE (3): X is Dab(diaminobutyric acid)
  MISC_FEATURE (6)..(7): X is Dab
  MISC_FEATURE (10): X is Dab
LCXLLXXLCX

SEQ ID NO: 27 - protein, 10 aa, Artificial Sequence
  synthetic peptide
  MISC_FEATURE (3): X is Dap(diaminopropionic acid)
  MISC_FEATURE (6)..(7): X is Dap
  MISC_FEATURE (10): X is Dap
LCXLLXXLCX

SEQ ID NO: 28 - protein, 10 aa, Artificial Sequence
  synthetic peptide
  MISC_FEATURE (3): X is hR(homoarginine)
  MISC_FEATURE (6)..(7): X is hR
  MISC_FEATURE (10): X is hR
LCXLLXXLCX

SEQ ID NO: 29 - protein, 10 aa, Artificial Sequence
  synthetic peptide
  MISC_FEATURE (3): X is norR(nor arginine)
  MISC_FEATURE (6)..(7): X is norR
  MISC_FEATURE (10): X is norR
LCXLLXXLCX

SEQ ID NO: 30 - protein, 10 aa, Artificial Sequence
  synthetic peptide
LCKLLRRLCR

SEQ ID NO: 31 - protein, 10 aa, Artificial Sequence
  synthetic peptide
LCRLLKRLCR

SEQ ID NO: 32 - protein, 10 aa, Artificial Sequence
  synthetic peptide
LCRLLRKLCR

SEQ ID NO: 33 - protein, 10 aa, Artificial Sequence
  synthetic peptide
LCRLLRRLCK

SEQ ID NO: 34 - protein, 10 aa, Artificial Sequence
  synthetic peptide
LCRLLRKLCK

SEQ ID NO: 35 - protein, 10 aa, Artificial Sequence
  synthetic peptide
LCRLLKRLCK

SEQ ID NO: 36 - protein, 10 aa, Artificial Sequence
  synthetic peptide
LCRLLKKLCR

SEQ ID NO: 37 - protein, 10 aa, Artificial Sequence
  synthetic peptide
LCKLLRRLCK

SEQ ID NO: 38 - protein, 10 aa, Artificial Sequence
  synthetic peptide
LCKLLRKLCR

SEQ ID NO: 39 - protein, 10 aa, Artificial Sequence
  synthetic peptide
LCKLLKRLCR

SEQ ID NO: 40 - protein, 10 aa, Artificial Sequence
  synthetic peptide
  MISC_FEATURE (9): X is Hcy(homocysteine)
LCKLLKKLXK

SEQ ID NO: 41 - protein, 10 aa, Artificial Sequence
  synthetic peptide
  MISC_FEATURE (2): X is Hcy
  MISC_FEATURE (9): X is Hcy
LXKLLKKLXK

SEQ ID NO: 42 - protein, 10 aa, Artificial Sequence
  synthetic peptide
  MISC_FEATURE (2): X is Hcy
LXRLLRRLCR

SEQ ID NO: 43 - protein, 10 aa, Artificial Sequence
  synthetic peptide
  MISC_FEATURE (9): X is Hcy
LCRLLRRLXR

SEQ ID NO: 44 - protein, 10 aa, Artificial Sequence
  synthetic peptide
  MISC_FEATURE (2): X is Hcy
  MISC_FEATURE (9): X is Hcy
LXRLLRRLXR

SEQ ID NO: 45 - protein, 10 aa, Artificial Sequence
  synthetic peptide
  MISC_FEATURE (2): X is U(selenocysteine)
  MISC_FEATURE (9): X is U
LXKLLKKLXK

SEQ ID NO: 46 - protein, 10 aa, Artificial Sequence
  synthetic peptide
  MISC_FEATURE (2): X is Pen(penicillamine)
  MISC_FEATURE (9): X is Pen
LXKLLKKLXK

SEQ ID NO: 47 - protein, 16 aa, Artificial Sequence
  synthetic peptide
  MISC_FEATURE (12): X is Hcy
LKKLCKLLKKLXKLAG

SEQ ID NO: 48 - protein, 16 aa, Artificial Sequence
  synthetic peptide
  MISC_FEATURE (5): X is Hcy
  MISC_FEATURE (12): X i sHcy
LKKLXKLLKKLXKLAG